European Patent Specification EP 3 858 977 B1, published February 28, 2024. Title: 一种用于预防和治疗代谢疾病的菌株及其应用. Applicant: 上海上药信谊药厂有限公司 上海市内分泌代谢病研究所. The sequence listing filed with the application follows.

SEQUENCE LISTING (1 sequence)

SEQ ID NO: 1 - DNA, 1421 bp, Akkermansia muciniphila
gaccccgtctaaccttaggaccctgcctccttgcggttggcttcagatacttcgggtgcgaccggcttccatgatgtgacgggcggtgtgtacaagacccgggaacgtattcacggcgccgtagctgatgcgccattactagcgattccggcttcgtgtaggcgggttgcagcctacagtccgaactgggcccagtttttaggatttcctccgcctcgcggcttcggccccctctgtactgggcattgtagtacgtgtgcagccctgggcataagggccatactgacctgacgtcgtccccaccttcctcccagttgatctgggcagtctcgccagagtccccaccttcacgtgctggtaactggcaacaggggttgcgctcgttgctggacttaaccaaacatctcacgacacgagctgacgacggccatgcagcacctgtgtaacgcctccgaagagtcgcatgctttcacatgttgttcattacatgtcaagcccaggtaaggttcttcgcgttgcatcgaattaagccacatactccaccgcttgtgcgggtccccgtcaatttctttgagttttaatcttgcgaccgtactccccaggcggcacgcttaacgcgttagctccggcacgcagggggtcgattccccgcacaccaagcgtgcaccgtttactgccaggactacaggggtatctaatccctttcgctcccctggccttcgtgcctcagcgtcagttaatgtccaggaacccgccttcgccacgagtgttcctctcgatatctacgcatttcactgctacaccgagaattccggttccccctccattactctagtctcgcagtatcatgtgccgtccgcgggttgagcccgcgcctttcacacacgacttacgaaacagcctacgcacgctttacgcccagtgattccgaacaacgcttgagacctctgtattaccgcggctgctggcacagagttagccgtctcttcctcttgtggtactatctttttaatttgctcccacatgacaggggtttacaatccgaagaccttcattcccccacgcggcgtcgcaccatcagggtttcccccattgtgaatgattctcgactgctgccacccgtaggtgtctggaccgtgtctcagttccagtgtggccggacatcctctcagaccggctacccgtcatcgccttggtgagccgttacctcaccaactaactaataggccgcgagcccatccccaagcgcattgctgctttaatctttcgatactatgcggtattaatcccagtttcccagggctatcccgctctcgggggcaggttactcacgtgttactcacccgtgcgccactagagaattattagcaagctagcaattctctcgttcgacttgcattctaagcaggccggccacggcc